European Patent Application EP 4 620 962 A1, published September 24, 2025. Title: Peptide having activities of hair growth promotion and hair loss inhibitory and uses thereof. Applicant: CAREGEN CO., LTD. Application WO. The sequence listing filed with the application follows.

SEQUENCE LISTING (20 sequences)

SEQ ID NO: 1 - DNA, 20 bp, synthetic construct
  source 1..20: mol_type = other DNA
ccagctattgtaacacctca

SEQ ID NO: 2 - DNA, 20 bp, synthetic construct
  source 1..20: mol_type = other DNA
ttcagatgtaggcagctgtc

SEQ ID NO: 3 - DNA, 25 bp, synthetic construct
  source 1..25: mol_type = other DNA
accagcagcgactctgaggaggaac

SEQ ID NO: 4 - DNA, 26 bp, synthetic construct
  source 1..26: mol_type = other DNA
tgaccctcttggcagcaggatagtcc

SEQ ID NO: 5 - DNA, 28 bp, synthetic construct
  source 1..28: mol_type = other DNA
accttcgttgccctctgtgccacagatg

SEQ ID NO: 6 - RNA, 21 nt, synthetic construct
  source 1..21: mol_type = other RNA
aggcccggaggcagtccgggt

SEQ ID NO: 7 - DNA, 20 bp, synthetic construct
  source 1..20: mol_type = other DNA
ggagccaaaagggtcatcat

SEQ ID NO: 8 - DNA, 20 bp, synthetic construct
  source 1..20: mol_type = other DNA
gtgatggcatggactgtggt

SEQ ID NO: 9 - DNA, 20 bp, synthetic construct
  source 1..20: mol_type = other DNA
gatcatcgagctgagacgca

SEQ ID NO: 10 - DNA, 20 bp, synthetic construct
  source 1..20: mol_type = other DNA
ctggccccagggtatctagt

SEQ ID NO: 11 - DNA, 20 bp, synthetic construct
  source 1..20: mol_type = other DNA
ccctcaaggatgccaggaac

SEQ ID NO: 12 - DNA, 19 bp, synthetic construct
  source 1..19: mol_type = other DNA
cactgctacctccggcaag

SEQ ID NO: 13 - DNA, 20 bp, synthetic construct
  source 1..20: mol_type = other DNA
ccaaatccgcaccaaggtca

SEQ ID NO: 14 - DNA, 21 bp, synthetic construct
  source 1..21: mol_type = other DNA
gtattgattgccaggaggggg

SEQ ID NO: 15 - DNA, 20 bp, synthetic construct
  source 1..20: mol_type = other DNA
cgcggcgtatccgtgtcctc

SEQ ID NO: 16 - DNA, 24 bp, synthetic construct
  source 1..24: mol_type = other DNA
agcctgttccgtctcaaacttggt

SEQ ID NO: 17 - DNA, 20 bp, synthetic construct
  source 1..20: mol_type = other DNA
cggtcaagtcggaaaattca

SEQ ID NO: 18 - DNA, 20 bp, synthetic construct
  source 1..20: mol_type = other DNA
gaggagctgggatgtggtaa

SEQ ID NO: 19 - DNA, 20 bp, synthetic construct
  source 1..20: mol_type = other DNA
caggactgggtgatggtgtc

SEQ ID NO: 20 - DNA, 20 bp, synthetic construct
  source 1..20: mol_type = other DNA
tctgagggtgagagcctgaa